European Patent Specification EP 3 877 056 B1, published July 2, 2025. Title: TEPOXALIN TARGETING OF ABCB1 OVEREXPRESSING CANCERS. Applicant: Broad Institute, Inc. Dana Farber Cancer Institute, Inc. The sequence listing filed with the application follows.

SEQUENCE LISTING (2 sequences)

SEQ ID NO: 1 - DNA, 4363 bp, Homo sapiens
gctcattcgagtagcggctcttccaagctcaaagaagcagaggccgctgttcgtttcctttaggtctttccactaaagtcggagtatcttcttccaaaatttcacgtcttggtggccgttccaaggagcgcgaggtcggaatggatcttgaaggggaccgcaatggaggagcaaagaagaagaacttttttaaactgaacaataaaagtgaaaaagataagaaggaaaagaaaccaactgtcagtgtattttcaatgtttcgctattcaaattggcttgacaagttgtatatggtggtgggaactttggctgccatcatccatggggctggacttcctctcatgatgctggtgtttggagaaatgacagatatctttgcaaatgcaggaaatttagaagatctgatgtcaaacatcactaatagaagtgatatcaatgatacagggttcttcatgaatctggaggaagacatgaccaggtatgcctattattacagtggaattggtgctggggtgctggttgctgcttacattcaggtttcattttggtgcctggcagctggaagacaaatacacaaaattagaaaacagttttttcatgctataatgcgacaggagataggctggtttgatgtgcacgatgttggggagcttaacacccgacttacagatgatgtctccaagattaatgaaggaattggtgacaaaattggaatgttctttcagtcaatggcaacatttttcactgggtttatagtaggatttacacgtggttggaagctaacccttgtgattttggccatcagtcctgttcttggactgtcagctgctgtctgggcaaagatactatcttcatttactgataaagaactcttagcgtatgcaaaagctggagcagtagctgaagaggtcttggcagcaattagaactgtgattgcatttggaggacaaaagaaagaacttgaaaggtacaacaaaaatttagaagaagctaaaagaattgggataaagaaagctattacagccaatatttctataggtgctgctttcctgctgatctatgcatcttatgctctggccttctggtatgggaccaccttggtcctctcaggggaatattctattggacaagtactcactgtattcttttctgtattaattggggcttttagtgttggacaggcatctccaagcattgaagcatttgcaaatgcaagaggagcagcttatgaaatcttcaagataattgataataagccaagtattgacagctattcgaagagtgggcacaaaccagataatattaagggaaatttggaattcagaaatgttcacttcagttacccatctcgaaaagaagttaagatcttgaagggtctgaacctgaaggtgcagagtgggcagacggtggccctggttggaaacagtggctgtgggaagagcacaacagtccagctgatgcagaggctctatgaccccacagaggggatggtcagtgttgatggacaggatattaggaccataaatgtaaggtttctacgggaaatcattggtgtggtgagtcaggaacctgtattgtttgccaccacgatagctgaaaacattcgctatggccgtgaaaatgtcaccatggatgagattgagaaagctgtcaaggaagccaatgcctatgactttatcatgaaactgcctcataaatttgacaccctggttggagagagaggggcccagttgagtggtgggcagaagcagaggatcgccattgcacgtgccctggttcgcaaccccaagatcctcctgctggatgaggccacgtcagccttggacacagaaagcgaagcagtggttcaggtggctctggataaggccagaaaaggtcggaccaccattgtgatagctcatcgtttgtctacagttcgtaatgctgacgtcatcgctggtttcgatgatggagtcattgtggagaaaggaaatcatgatgaactcatgaaagagaaaggcatttacttcaaacttgtcacaatgcagacagcaggaaatgaagttgaattagaaaatgcagctgatgaatccaaaagtgaaattgatgccttggaaatgtcttcaaatgattcaagatccagtctaataagaaaaagatcaactcgtaggagtgtccgtggatcacaagcccaagacagaaagcttagtaccaaagaggctctggatgaaagtatacctccagtttccttttggaggattatgaagctaaatttaactgaatggccttattttgttgttggtgtattttgtgccattataaatggaggcctgcaaccagcatttgcaataatattttcaaagattataggggtttttacaagaattgatgatcctgaaacaaaacgacagaatagtaacttgttttcactattgtttctagcccttggaattatttcttttattacatttttccttcagggtttcacatttggcaaagctggagagatcctcaccaagcggctccgatacatggttttccgatccatgctcagacaggatgtgagttggtttgatgaccctaaaaacaccactggagcattgactaccaggctcgccaatgatgctgctcaagttaaaggggctataggttccaggcttgctgtaattacccagaatatagcaaatcttgggacaggaataattatatccttcatctatggttggcaactaacactgttactcttagcaattgtacccatcattgcaatagcaggagttgttgaaatgaaaatgttgtctggacaagcactgaaagataagaaagaactagaaggttctgggaagatcgctactgaagcaatagaaaacttccgaaccgttgtttctttgactcaggagcagaagtttgaacatatgtatgctcagagtttgcaggtaccatacagaaactctttgaggaaagcacacatctttggaattacattttccttcacccaggcaatgatgtatttttcctatgctggatgtttccggtttggagcctacttggtggcacataaactcatgagctttgaggatgttctgttagtattttcagctgttgtctttggtgccatggccgtggggcaagtcagttcatttgctcctgactatgccaaagccaaaatatcagcagcccacatcatcatgatcattgaaaaaacccctttgattgacagctacagcacggaaggcctaatgccgaacacattggaaggaaatgtcacatttggtgaagttgtattcaactatcccacccgaccggacatcccagtgcttcagggactgagcctggaggtgaagaagggccagacgctggctctggtgggcagcagtggctgtgggaagagcacagtggtccagctcctggagcggttctacgaccccttggcagggaaagtgctgcttgatggcaaagaaataaagcgactgaatgttcagtggctccgagcacacctgggcatcgtgtcccaggagcccatcctgtttgactgcagcattgctgagaacattgcctatggagacaacagccgggtggtgtcacaggaagagattgtgagggcagcaaaggaggccaacatacatgccttcatcgagtcactgcctaataaatatagcactaaagtaggagacaaaggaactcagctctctggtggccagaaacaacgcattgccatagctcgtgcccttgttagacagcctcatattttgcttttggatgaagccacgtcagctctggatacagaaagtgaaaaggttgtccaagaagccctggacaaagccagagaaggccgcacctgcattgtgattgctcaccgcctgtccaccatccagaatgcagacttaatagtggtgtttcagaatggcagagtcaaggagcatggcacgcatcagcagctgctggcacagaaaggcatctatttttcaatggtcagtgtccaggctggaacaaagcgccagtgaactctgactgtatgagatgttaaatactttttaatatttgtttagatatgacatttattcaaagttaaaagcaaacacttacagaattatgaagaggtatctgtttaacatttcctcagtcaagttcagagtcttcagagacttcgtaattaaaggaacagagtgagagacatcatcaagtggagagaaatcatagtttaaactgcattataaattttataacagaattaaagtagattttaaaagataaaatgtgtaattttgtttatattttcccatttggactgtaactgactgccttgctaaaagattatagaagtagcaaaaagtattgaaatgtttgcataaagtgtctataataaaactaaactttcatgtga

SEQ ID NO: 2 - protein, 1280 aa, Homo sapiens
MDLEGDRNGGAKKKNFFKLNNKSEKDKKEKKPTVSVFSMFRYSNWLDKLYMVVGTLAAIIHGAGLPLMMLVFGEMTDIFANAGNLEDLMSNITNRSDINDTGFFMNLEEDMTRYAYYYSGIGAGVLVAAYIQVSFWCLAAGRQIHKIRKQFFHAIMRQEIGWFDVHDVGELNTRLTDDVSKINEGIGDKIGMFFQSMATFFTGFIVGFTRGWKLTLVILAISPVLGLSAAVWAKILSSFTDKELLAYAKAGAVAEEVLAAIRTVIAFGGQKKELERYNKNLEEAKRIGIKKAITANISIGAAFLLIYASYALAFWYGTTLVLSGEYSIGQVLTVFFSVLIGAFSVGQASPSIEAFANARGAAYEIFKIIDNKPSIDSYSKSGHKPDNIKGNLEFRNVHFSYPSRKEVKILKGLNLKVQSGQTVALVGNSGCGKSTTVQLMQRLYDPTEGMVSVDGQDIRTINVRFLREIIGVVSQEPVLFATTIAENIRYGRENVTMDEIEKAVKEANAYDFIMKLPHKFDTLVGERGAQLSGGQKQRIAIARALVRNPKILLLDEATSALDTESEAVVQVALDKARKGRTTIVIAHRLSTVRNADVIAGFDDGVIVEKGNHDELMKEKGIYFKLVTMQTAGNEVELENAADESKSEIDALEMSSNDSRSSLIRKRSTRRSVRGSQAQDRKLSTKEALDESIPPVSFWRIMKLNLTEWPYFVVGVFCAIINGGLQPAFAIIFSKIIGVFTRIDDPETKRQNSNLFSLLFLALGIISFITFFLQGFTFGKAGEILTKRLRYMVFRSMLRQDVSWFDDPKNTTGALTTRLANDAAQVKGAIGSRLAVITQNIANLGTGIIISFIYGWQLTLLLLAIVPIIAIAGVVEMKMLSGQALKDKKELEGSGKIATEAIENFRTVVSLTQEQKFEHMYAQSLQVPYRNSLRKAHIFGITFSFTQAMMYFSYAGCFRFGAYLVAHKLMSFEDVLLVFSAVVFGAMAVGQVSSFAPDYAKAKISAAHIIMIIEKTPLIDSYSTEGLMPNTLEGNVTFGEVVFNYPTRPDIPVLQGLSLEVKKGQTLALVGSSGCGKSTVVQLLERFYDPLAGKVLLDGKEIKRLNVQWLRAHLGIVSQEPILFDCSIAENIAYGDNSRVVSQEEIVRAAKEANIHAFIESLPNKYSTKVGDKGTQLSGGQKQRIAIARALVRQPHILLLDEATSALDTESEKVVQEALDKAREGRTCIVIAHRLSTIQNADLIVVFQNGRVKEHGTHQQLLAQKGIYFSMVSVQAGTKRQ